European Patent Specification EP 4 073 264 B1, published March 20, 2024. Title: Method for whole genome sequencing of picogram quantities of DNA. Applicant: Oxford University Innovation Limited. The sequence listing filed with the application follows.

SEQUENCE LISTING (22 sequences)

SEQ ID NO: 1 - DNA, 52 bp, Artificial Sequence
  indexed looped-adapter
agatcggaagagcacacgtctgaactuccctacacgacgctcttccgatctt

SEQ ID NO: 2 - DNA, 62 bp, Artificial Sequence
  Row indexing primer
aatgatacggcgaccaccgagatctacacacactctttccctacacgacgctcttccgatct

SEQ ID NO: 3 - DNA, 58 bp, Artificial Sequence
  row indexing primer
caagcagaagacggcatacgagatgtgactggagttcagacgtgtgctcttccgatct

SEQ ID NO: 4 - DNA, 23 bp, Homo sapiens
tgatcgcttccgagcaataagaa

SEQ ID NO: 5 - DNA, 23 bp, Homo sapiens
ccttatttctgatgctcttagat

SEQ ID NO: 6 - DNA, 23 bp, Homo sapiens
gtatcagtcagccagaaaaaagg

SEQ ID NO: 7 - DNA, 42 bp, Homo sapiens
tttattgaagtttgttttcctctttgatcctaccactttttt

SEQ ID NO: 8 - DNA, 42 bp, Homo sapiens
aagccaatgtattgatcgcttccgagcaataagaatagtgat

SEQ ID NO: 9 - DNA, 42 bp, Homo sapiens
gttgttgtttgccaagctaatctgcctggttttatttatatc

SEQ ID NO: 10 - DNA, 42 bp, Homo sapiens
aagtctacattaaacaatgatcacatctaaagctttatcttt

SEQ ID NO: 11 - DNA, 42 bp, Homo sapiens
ctcatatataaagccttatttctgatgctcttagatttctga

SEQ ID NO: 12 - DNA, 42 bp, Homo sapiens
gggactacagatgtgtgccatcacacccagctagttttttgt

SEQ ID NO: 13 - DNA, 42 bp, Homo sapiens
tgcataggtataggtatcagtcagccagaaaaaaggactttg

SEQ ID NO: 14 - DNA, 42 bp, Homo sapiens
gtatatatacaaatactttgtccatttaaaaaattaggttat

SEQ ID NO: 15 - DNA, 42 bp, Homo sapiens
cctatatagactaacatggatctaactttttgactatcttcc

SEQ ID NO: 16 - DNA, 42 bp, Homo sapiens
gaaatgctttgtgaaatatgtcaacatactggttgcaaatgc

SEQ ID NO: 17 - DNA, 42 bp, Homo sapiens
gagtatggctatctatacctgccttttaagtttgaaactaac

SEQ ID NO: 18 - DNA, 42 bp, Homo sapiens
gtctttcctctctctgtccttccccgaaagtctactcgggtg

SEQ ID NO: 19 - DNA, 42 bp, Homo sapiens
ggcatgatcactgcagcctctctgcttcccagattcaagtga

SEQ ID NO: 20 - DNA, 42 bp, Homo sapiens
cattaggggctggacactcatcgagatgacctgcctacaaat

SEQ ID NO: 21 - DNA, 42 bp, Homo sapiens
gattgaaactgtccatttaatctccttcctcccattatcaat

SEQ ID NO: 22 - DNA, 42 bp, Homo sapiens
tacctatttatctatatatttcaacttataaaactttctttc